European Patent Application EP 4 600 371 A1, published August 13, 2025. Title: Cell-free glycosylation of peptides and proteins. Applicant: ETH Zurich. Application EP. The sequence listing filed with the application follows.

SEQUENCE LISTING (38 sequences)

SEQ ID NO: 1 - skipped

SEQ ID NO: 2 - protein, 5 aa, unidentified
  SITE 1: note = X = D or E
XANYT

SEQ ID NO: 3 - protein, 5 aa, unidentified
  SITE 2: note = X = A or V
LXNYT

SEQ ID NO: 4 - protein, 40 aa, synthetic construct
  CARBOHYD 3..7: note = glycosylation sequon
  CARBOHYD 18..22: note = glycosylation sequon
  CARBOHYD 33..37: note = glycosylation sequon
GSDANYTYTQSEKSAASEANYTYSAEGRGSESDANYTYTK

SEQ ID NO: 5 - protein, 41 aa, synthetic construct
  CARBOHYD 3..7: note = glycosylation sequon
  CARBOHYD 18..22: note = glycosylation sequon
  CARBOHYD 33..37: note = glycosylation sequon
GSLANYTYTQSEKSDASLVNYTYSSEGRGSESLANYTYTEK

SEQ ID NO: 6 - protein, 203 aa, synthetic construct
  SITE 33: note = cysteine residue for labelling with fluorophore
  SITE 36: note = cysteine residues for labelling with fluorophore
  SITE 163: note = cysteine residue for labelling with fluorophore
  CARBOHYD 166..170: note = glycosylation sequon
  CARBOHYD 181..185: note = glycosylation sequon
  CARBOHYD 196..200: note = glycosylation sequon
MSDKIIHLTDDSFDTDVLKADGAILVDFWAEWCGPCKMIAPILDEIADEYQGKLTVAKLNIDQNPGTAPKYGIRGIPTLLLFKNGEVAATKVGALSKGQLKEFLDANLAGSGSGHMHHHHHHHHSSGLVPRGSGMKETAAAKFERQHMDSPDLGTENLYFQSCGSDANYTYTQSEKSAASEANYTYSAEGRGSESDANYTYTK

SEQ ID NO: 7 - protein, 204 aa, synthetic construct
  SITE 33: note = cysteine residue for labelling with fluorophore
  SITE 36: note = cysteine residue for labelling with fluorophore
  SITE 163: note = cysteine residue for labelling with fluorophore
  CARBOHYD 166..170: note = glycosylation sequon
  CARBOHYD 181..185: note = glycosylation sequon
  CARBOHYD 196..200: note = glycosylation sequon
MSDKIIHLTDDSFDTDVLKADGAILVDFWAEWCGPCKMIAPILDEIADEYQGKLTVAKLNIDQNPGTAPKYGIRGIPTLLLFKNGEVAATKVGALSKGQLKEFLDANLAGSGSGHMHHHHHHHHSSGLVPRGSGMKETAAAKFERQHMDSPDLGTENLYFQSCGSLANYTYTQSEKSDASLVNYTYSSEGRGSESLANYTYTEK

SEQ ID NO: 8 - DNA, 2421 bp, Trypanosoma brucei
  source 1..2421: mol_type = genomic DNA
atggggagcgctatgggcaccaagggtggaaaggtggccgtgaccaagggttccgctcagtctgacggtgctggcgagggtggcatgtccaaggctaagtcctccaccaccttcgtggctaccggtggtggttccctgcctgcttgggctctgaaggctgtgtccaccatcgtgtccgctgtgatcctgatctactccgtgcaccgtgcttacgacatccgtctgacctccgtgcgtctgtacggcgagctgatccacgagttcgacccctggttcaactaccgtgctacccagtacctgtccgacaacggctggcgcgctttcttccagtggtacgactacatgtcctggtaccccctaggccgtcctgtgggcaccaccatcttccccggaatgcagctgaccggtgtcgctatccaccgtgtgctcgagatgctgggtcgtggaatgtccatcaacaacatctgcgtgtacatccccgcctggttcggttctatcgctaccgtcctggctgctctgatcgcttacgagtcctccaactccctgtccgtgatggctttcaccgcttacttcttctccatcgtgcctgctcacctgatgcgttctatggctggcgaattcgacaacgagtgtgtggctatggctgctatgctgctgaccttctatatgtgggtccgctccctgaggtcctcctcctcttggcctatcggcgccctggctggtgtcgcttacggttacatggtgtccacctggggcggttacatcttcgtgctgaacatggtggctttccacgcttccgtgtgcgtgctgctggactgggctcgtggtacttactccgtgtccctgctgcgcgcttactccctgttcttcgtgatcggcaccgctctggctatctgcgtgccccctgtggaatggaccccattccgttccctggaacagctgactgctctgttcgtgttcgttttcatgtgggctctgcactactccgagtacctgcgcgagcgtgctcgtgctcctatccactcctccaaggctctgcagatccgtgctcgtatcttcatgggcaccctgtctctgctgctgatcgtggcttccctgctggctcccttcggtttcttcaagcctaccgcttaccgcgtgcgcgccctgttcgtgaagcacacccgtaccggcaacccactagtggactccgtggctgagcaccgtcctaccaccgctggtgcttacctgcgctacttccacgtctgctaccctctgtggggttgcggtggcctgtccatgctggtgttcatgaagaaggaccgttggcgcgccatcgtgttcctcgcttccctgtccaccgtgaccatgtacttctccgctcgtatgtcccgcctgctgctgctcgctggtcctgctgctactgcatgcgctggcatgttcatcggtggactgttcgacctggctctgtcccagttcggcgacctgcgttcccctaaggacgcttccggcgactctgaccccgctggtggttctaagcgtgctaagggcaaggtggtcaacgagccctccgagcgcgctatcttctcccaccgttggttccagcgtctggtgcagtctctgcccgtgcccttaagacgtggtatcgctgtggtggtgctcgtgtgcctgttcgctaaccctatgcgccactccttcgaaaagtcctgcgagaagatggctcacgctctgtcctccccccgtatcatcgctgtgaccgacctgcctaacggcgagcgtgtgctggctgacgactactacgtgtcctacctgtggctgcgtaacaacacccccgaggacgctcgtatcctgtcttggtgggactacggttaccagatcaccggtatcggcaaccgtaccaccctggccgacggaaacacgtggtcccacaagcacatcgctaccatcggcaagatgctgacctcccccgtgaaggaatcccacgctctgatccgtcacctggctgactacgtgctgatctgggctggttacgacggttccgacctgctgaagtccccccacatggctcgcatcggcaactccgtataccgtgacatgtgctccgaggacgaccccctgtgccgtcagttcggattctactctggcgacctgaacaagcccacccccatgatgcagcgctccctgctgtacaacctgcaccgtttcggcaccgacggtggcaagacccagctggacaagaacatgttccagctggcttatgtgtcgaagtacggcctggtcaagatctacaaagtgatgaacgtgtccgaggaatccaaggcttgggtggccgaccccaagaaccgtgtgtgcgaccctcctggttcctggatctgcgctggccagtacccccctgctaaggaaatccaagacatgctggctaagcgcttccactacgagtaa

SEQ ID NO: 9 - protein, 806 aa, Trypanosoma brucei
MGSAMGTKGGKVAVTKGSAQSDGAGEGGMSKAKSSTTFVATGGGSLPAWALKAVSTIVSAVILIYSVHRAYDIRLTSVRLYGELIHEFDPWFNYRATQYLSDNGWRAFFQWYDYMSWYPLGRPVGTTIFPGMQLTGVAIHRVLEMLGRGMSINNICVYIPAWFGSIATVLAALIAYESSNSLSVMAFTAYFFSIVPAHLMRSMAGEFDNECVAMAAMLLTFYMWVRSLRSSSSWPIGALAGVAYGYMVSTWGGYIFVLNMVAFHASVCVLLDWARGTYSVSLLRAYSLFFVIGTALAICVPPVEWTPFRSLEQLTALFVFVFMWALHYSEYLRERARAPIHSSKALQIRARIFMGTLSLLLIVASLLAPFGFFKPTAYRVRALFVKHTRTGNPLVDSVAEHRPTTAGAYLRYFHVCYPLWGCGGLSMLVFMKKDRWRAIVFLASLSTVTMYFSARMSRLLLLAGPAATACAGMFIGGLFDLALSQFGDLRSPKDASGDSDPAGGSKRAKGKVVNEPSERAIFSHRWFQRLVQSLPVPLRRGIAVVVLVCLFANPMRHSFEKSCEKMAHALSSPRIIAVTDLPNGERVLADDYYVSYLWLRNNTPEDARILSWWDYGYQITGIGNRTTLADGNTWSHKHIATIGKMLTSPVKESHALIRHLADYVLIWAGYDGSDLLKSPHMARIGNSVYRDMCSEDDPLCRQFGFYSGDLNKPTPMMQRSLLYNLHRFGTDGGKTQLDKNMFQLAYVSKYGLVKIYKVMNVSEESKAWVADPKNRVCDPPGSWICAGQYPPAKEIQDMLAKRFHYE

SEQ ID NO: 10 - DNA, 2481 bp, Trypanosoma brucei
  source 1..2481: mol_type = genomic DNA
atggggagcgctatgggtacaaaaggtggcaaggtggccgtgaccaagggttccgctcaatctgatggtgctggcgaaggtggcatgtccaaggctaagtcctccaccaccttcgtggctaccggtggtggttctttgcctgcttgggctctgaaggctgtgtccaccatcgtgtccgctgtgatcctgatctactccgtgcaccgtgcttacgacatccgtctgacctccgtccgtctgtacggcgagctgatccacgaattcgacccctggttcaactaccgtgctacccagtacctgtccgacaacggatggcgcgctttcttccagtggtacgactatatgtcctggtatcccctgggtcgtcccgtgggcactactatcttccctggaatgcagctgaccggtgtcgctatccaccgtgtgctggaaatgctcggtcgtggaatgtccatcaacaacatctgcgtgtacatccccgcttggtttggttctatcgctaccgtcctggctgctctgatcgcttacgagtcctccaactccttaagtgtgatggccttcaccgcctactttttctccatcgtgcctgctcacctgatgcgttctatggctggcgagttcgacaacgagtgtgtggctatggctgctatgctgctgaccttctatatgtgggtccgatctctgcgctcctcctcctcttggcctattggtgctctggctggtgtcgcttacggttacatggtgtctacctggggcggttacatcttcgtgctgaacatggtggctttccacgcttccgtgtgcgtgctgttggattgggctcgtggcacctactctgtgtccctgctgagggcttactccctgttcttcgtgatcggcaccgctctggctatctgcgtgccacctgttgagtggaccccattccgttccttggagcagctgactgctctgttcgtgttcgttttcatgtgggctctgcactactccgagtacctgcgtgaacgtgctcgtgctcctatccactcctccaaggctctgcagatccgtgctcgtatcttcatgggtactctgtctctgctgctgatcgtggctatctacctgttctccaccggttacttccgtcctttctcctctcgtgtgcgcgccctgttcgtgaagcacaccagaactggcaacccactagtggactccgtggctgagcaccatcctgcttccaacgacgacttcttcggttacctgcacgtgtgctacaacggctggattatcggcttcttctttatgtccgtgtcctgcttcttccactgtactcccggaatgtccttcctgctgctgtactccatcctggcttactacttcagcctgaagatgtcccgtctgctgctcctgtcagctcccgtggcttctatcctgaccggttacgtcgtgggttccatcgtggacttggctgccgattgcttcgctgcttccggtactgagcacgctgactccaaagaacaccaaggcaaggctcgtggaaagggccagaaagagcagatcaccgtcgagtgcggttgtcacaaccccttctacaagctgtggtgcaactccttctcttcccgtctggtcgtgggcaagttcttcgtcgtggtggtgctcgctatctgtggtcccaccttcctagggtccaacctgcgcatctactctgagcagttcgccgactccatgtcctcacctcagatcatcatgcgtgctaccgtcggtggtcgtcgcgtgatcttggacgactactacgtgtcctacctgtggctgcgtaacaacacccctgaggacgctcgtatcctgtcttggtgggactacggttaccagatcactggtatcggcaaccgtaccactctggctgacggcaacacttggaaccacgagcacattgctaccatcggcaagatgctgacctctcctgtgaaagagtcccacgctctgatccgtcacctggctgactacgtgctgatctgggctggttacgacggttccgacctgctgaagtcccctcacatggctcgtatcggaaactccgtgtaccgcgacatctgctccgaggacgaccctctgtgcacccagttcggtttctactccggcgacttctccaagcctactcctatgatgcagcgttccctgctgtacaacctgcaccgtttcggtactgacggtggcaagacccagctggacaaaaacatgttccagctggcctacgtttcgaagtacggcctggtcaagatctacaaagtgatgaacgtgtccgaggaatccaaggcttgggtcgccgatcctaagaaccgtgtgtgcgaccctcctggttcttggatctgcgctggacagtaccctcctgctaaagaaatccaggacatgctggctaagcgcatcgactacgagcagctcgaggacttcaaccgtcgcaaccgttccgacgcttactaccgcgcttacatgcgtcagatgggctaa

SEQ ID NO: 11 - protein, 826 aa, Trypanosoma brucei
  SITE 84: note = residue predicted to be involved in peptide binding, predicted catalytic residue
  SITE 395: note = residues predicted to be involved in peptide binding; predicted catalytic residue
  SITE 604..606: note = site predicted to be involved in peptide binding
  SITE 374: note = residue predicted to be invloved in lipid-linked oligosaccharide (LLO) binnding, predicted to be involved in pyrophosphate recognition
  SITE 453: note = residue predicted to be invloved in lipid-linked oligosaccharide (LLO) binnding, predicted to be involved in pyrophosphate recognition
  SITE 622..625: note = residue predicted to be invloved in lipid-linked oligosaccharide (LLO) binnding, predicted to be involved in GlcNAc2 binding
MGSAMGTKGGKVAVTKGSAQSDGAGEGGMSKAKSSTTFVATGGGSLPAWALKAVSTIVSAVILIYSVHRAYDIRLTSVRLYGELIHEFDPWFNYRATQYLSDNGWRAFFQWYDYMSWYPLGRPVGTTIFPGMQLTGVAIHRVLEMLGRGMSINNICVYIPAWFGSIATVLAALIAYESSNSLSVMAFTAYFFSIVPAHLMRSMAGEFDNECVAMAAMLLTFYMWVRSLRSSSSWPIGALAGVAYGYMVSTWGGYIFVLNMVAFHASVCVLLDWARGTYSVSLLRAYSLFFVIGTALAICVPPVEWTPFRSLEQLTALFVFVFMWALHYSEYLRERARAPIHSSKALQIRARIFMGTLSLLLIVAIYLFSTGYFRPFSSRVRALFVKHTRTGNPLVDSVAEHHPASNDDFFGYLHVCYNGWIIGFFFMSVSCFFHCTPGMSFLLLYSILAYYFSLKMSRLLLLSAPVASILTGYVVGSIVDLAADCFAASGTEHADSKEHQGKARGKGQKEQITVECGCHNPFYKLWCNSFSSRLVVGKFFVVVVLAICGPTFLGSNLRIYSEQFADSMSSPQIIMRATVGGRRVILDDYYVSYLWLRNNTPEDARILSWWDYGYQITGIGNRTTLADGNTWNHEHIATIGKMLTSPVKESHALIRHLADYVLIWAGYDGSDLLKSPHMARIGNSVYRDICSEDDPLCTQFGFYSGDFSKPTPMMQRSLLYNLHRFGTDGGKTQLDKNMFQLAYVSKYGLVKIYKVMNVSEESKAWVADPKNRVCDPPGSWICAGQYPPAKEIQDMLAKRIDYEQLEDFNRRNRSDAYYRAYMRQMG

SEQ ID NO: 12 - DNA, 411 bp, Streptococcus mutans
  source 1..411: mol_type = other DNA
atgcccatggacttacgtgacaataaacagtcccagaaaaagtggaagaatcgtactttaacgtcctcacttgagttcgctttaacaggaatcttcacagctttcaaggaggagcgtaatatgaagaaacatgcagtttccgcattacttgccgtaatcgccgggcttgttttcaaagtctccgttatcgagtggttatttctgttattatcgatttttttggtcatcacttttgaaattgtaaactccgctattgagaatgtcgtggacctggcgagcgattatcatttctctatgttagcgaagaacgctaaggatatggcggctggtgcggtgttagttatctctggattcgccgccttgactggcttgattatttttgtgccaaaaatctggtttcttctttttcat

SEQ ID NO: 13 - protein, 137 aa, Streptococcus mutans
MPMDLRDNKQSQKKWKNRTLTSSLEFALTGIFTAFKEERNMKKHAVSALLAVIAGLVFKVSVIEWLFLLLSIFLVITFEIVNSAIENVVDLASDYHFSMLAKNAKDMAAGAVLVISGFAALTGLIIFVPKIWFLLFH

SEQ ID NO: 14 - DNA, 984 bp, Sulfolobus acidocaldarius
  source 1..984: mol_type = other DNA
atgctggttagcctgctgggtattctgctgagcgttattgttggttttgttgttaccctgattagcaccaaatgggttattggtctgtgtaagaaacgtggttttaccggcaaagatatcaacaaactgaccaaagatgatgtgccggttttaggtggtattggtattgttgcaggttttgtggcaggtagctttacctttctgctgaccagctataacctgagtccgggtattgaaaatgttgttgttagcattctgctgtcgagcctgattattggttttctgggtctgctggatgatatcttcaatattagccaggcaacccgtgcatttctgccgatttttgcaagcattccgctgattctgtatagcgttggtcataccattattagcattccgtttctgggcaaagtgaactttggcatcctgttctatattatcattctgcctgcaacactgaccattaccgcaaatgcctttaacatgctggaaggtctgaatggtttaggtgcaggtatgggtctgattatggcactggccctggcatatattggcctgaaaagcggtggtacaagcttttatgcaggtattgtgagcattattctggccagcgttctgtttggctttctgatctttaacttctatcctgccaaaacctttccgggtaatattggcacctattttatcggtagcgtgattggtagcattggtattagcggttatatgtataccgcactgttctttctgtatctgccgtatgttattgagtttgtgctgaaagcaaaaacccgctttaaaggtgttagcttcggcaaaattgatgatcagggttatctgcattgggatagcaaaccgaatagtctgacccatattgttatgcgcattggcaaattcaaagaataccatatcgtgctgattatctggggcattgaaattctgtttgcaattctggcagttgtgtttcagaccgttaccattaccatt

SEQ ID NO: 15 - protein, 328 aa, Sulfolobus acidocaldarius
MLVSLLGILLSVIVGFVVTLISTKWVIGLCKKRGFTGKDINKLTKDDVPVLGGIGIVAGFVAGSFTFLLTSYNLSPGIENVVVSILLSSLIIGFLGLLDDIFNISQATRAFLPIFASIPLILYSVGHTIISIPFLGKVNFGILFYIIILPATLTITANAFNMLEGLNGLGAGMGLIMALALAYIGLKSGGTSFYAGIVSIILASVLFGFLIFNFYPAKTFPGNIGTYFIGSVIGSIGISGYMYTALFFLYLPYVIEFVLKAKTRFKGVSFGKIDDQGYLHWDSKPNSLTHIVMRIGKFKEYHIVLIIWGIEILFAILAVVFQTVTITI

SEQ ID NO: 16 - DNA, 981 bp, Sulfolobus acidocaldarius
  source 1..981: mol_type = other DNA
atgattgataacccgctgctgattattgcaagcggtggtggtcataccggttttgcacgtgccattgcagaatatctgccgtttaaaccggattttgtgattccggaaaatgaccgctttagcaaagatatgctgctggattatgcacgcaaactgtattatgtgaagaaaggtaaagatccaggccagggtaatattgttctgatgcgtaatttcctgaaaatcatcatcgaaagcggcaaaatcccgaaatatctggcaaccattgcaaccggtagtaatcatagcctgattccggcaatgttccagaaaatcaaaggtagcgcactgtatgttaccgaaagccaggatcgcattattacccgtggtaaaaccgttagcgttctgagcaaatttagccgtcatgtttttctgcattggaacgaacagaaaggcctgtatgataatggtgttgttgttggtccgattgtggaaaaaccgaaatacaaaagcgagaacaaaggctatattctggttaccaccggtagcatgggttttaagaaactgtttgatagcctgctgaatctgcgtggcaattacaaattcgttattcagaccggtaaagttgatccgacaccgtatattgaaaagaaacctgattggagcttctttagcttcgataaagatatcgaacgctatattgcaaatgccgaactggttattacccatcagggcaaaaccgcaatggaaagcgttgttatgtatggtaaaccgaccatcatcgtgtataacaaagattggaaaagcgcaaccaccaaacaggataccattctgtatagcaaaattctgggtgcaacctttctggatgatccgagcacctgggatagcattaaagttctggaagatagcattcagaatgtgcgtaaaccgaaccagtttgaaattggcaccccgaaactgatcgatattattctgagcgaactggcagaatttctgcgcgaa

SEQ ID NO: 17 - protein, 327 aa, Sulfolobus alphaportoglobovirus 1
MIDNPLLIIASGGGHTGFARAIAEYLPFKPDFVIPENDRFSKDMLLDYARKLYYVKKGKDPGQGNIVLMRNFLKIIIESGKIPKYLATIATGSNHSLIPAMFQKIKGSALYVTESQDRIITRGKTVSVLSKFSRHVFLHWNEQKGLYDNGVVVGPIVEKPKYKSENKGYILVTTGSMGFKKLFDSLLNLRGNYKFVIQTGKVDPTPYIEKKPDWSFFSFDKDIERYIANAELVITHQGKTAMESVVMYGKPTIIVYNKDWKSATTKQDTILYSKILGATFLDDPSTWDSIKVLEDSIQNVRKPNQFEIGTPKLIDIILSELAEFLRE

SEQ ID NO: 18 - DNA, 1350 bp, Saccharomyces cerevisiae
  source 1..1350: mol_type = other DNA
atgtttttggaaattcctcggtggttacttgccttaataatattatacctttccataccgttagtggtttattatgttataccctacttgttttatggcaacaagtcgaccaaaaaaaggatcatcatatttgtgctgggtgatgtaggacactctccaaggatatgctatcacgctataagtttcagtaagttaggttggcaagtcgagctatgcggttatgtggaggacactctacccaaaattatttccagtgatccaaatatcaccgtccatcatatgtcaaacttgaaaagaaagggaggcggaacatcagttatatttatggtaaagaaggtgctttttcaagttttaagtattttcaaattactttgggaattgagaggaagcgattacatactagttcaaaatccaccgagcatacccattcttccgattgctgtgctatacaagttgaccggttgtaaactaattattgattggcacaatctagcatattcgatattgcaactaaaatttaaaggaaacttttaccatcctttagtgttgatatcttacatggtagagatgatattcagcaaatttgctgattataacttgactgttactgaagcaatgaggaaatatttaattcaaagctttcacttgaatccaaagagatgtgctgttctctacgaccgcccggcttcccaatttcaacctttggcaggtgacatttctcgtcaaaaagccctaactaccaaagcctttataaagaattatattcgcgatgattttgatacagaaaaaggcgataaaattattgtgacttcaacatcattcacccctgatgaagatattggtattttattaggtgccctaaagatttacgaaaactcttatgtcaaatttgattcaagtttgcctaagatcttgtgttttataacgggtaaaggaccactaaaggagaaatatatgaagcaagtagaagaatatgactggaagcgctgtcaaatcgaatttgtgtggttgtcagcagaggattacccaaagttattacaattatgcgattacggagtttccctgcatacttcaagttcagggttggacctgccaatgaaaattttagatatgtttggctcaggtcttcctgttattgcaatgaactatccagtgcttgacgaattagtacaacacaatgtaaatgggttaaaatttgttgatagaagggagcttcatgaatctctgatttttgctatgaaagatgctgatttataccaaaaattgaagaaaaatgtaacgcaggaagctgagaacagatggcaatcaaattgggaacgaacaatgagagatttgaagctaattcattga

SEQ ID NO: 19 - protein, 449 aa, Saccharomyces cerevisiae
MFLEIPRWLLALIILYLSIPLVVYYVIPYLFYGNKSTKKRIIIFVLGDVGHSPRICYHAISFSKLGWQVELCGYVEDTLPKIISSDPNITVHHMSNLKRKGGGTSVIFMVKKVLFQVLSIFKLLWELRGSDYILVQNPPSIPILPIAVLYKLTGCKLIIDWHNLAYSILQLKFKGNFYHPLVLISYMVEMIFSKFADYNLTVTEAMRKYLIQSFHLNPKRCAVLYDRPASQFQPLAGDISRQKALTTKAFIKNYIRDDFDTEKGDKIIVTSTSFTPDEDIGILLGALKIYENSYVKFDSSLPKILCFITGKGPLKEKYMKQVEEYDWKRCQIEFVWLSAEDYPKLLQLCDYGVSLHTSSSGLDLPMKILDMFGSGLPVIAMNYPVLDELVQHNVNGLKFVDRRELHESLIFAMKDADLYQKLKKNVTQEAENRWQSNWERTMRDLKLIH

SEQ ID NO: 20 - DNA, 1200 bp, Caenorhabditis elegans
  source 1..1200: mol_type = other DNA
atggtccgtgttaccattcttcatccagacctggggattgggggtgcggagcgtttaatcgttgatgcggctgtaggtttacaggaccgcggtcacagcgtgcgtatttttactaatcaatactctcgctcgcactgttttcaagaaacgctggatttagatatctgcactgtagtcccatggattcctcgttcaatcttcggcaagggccacgctttatgtgcgtacttaaagatgatcattgctgcgctgtatatcgtgatctaccataaggataccgacgttattctgtcagactccgtgagcgctagccaatttgtgcttcgccatttttctaaagcaaaacttgttttttactgccatttcccagatcgcttgcttacgaaacgtgatgggaatttaaaggcgttctaccgtaatatcattgactggattgaagagtatacgacggggcttgctgacgtcatttgcgttaattccaacttcactaaaaatgttgtacgcgagaccttcaaatctttggcctcgcaggaactgaccgtcttgtaccccagcttgaacacggagttcttcgatagcatcgaggcgagtgatgatttcggcgaggagattcctcgcggcaccaaatatgtctttacgagtttaaatcgtttcgaacgtaaaaagaacattgttttagcccttgatgccttcgaaaaactgaaatctaacttgcctgcagatgagtttagtcaatgccatttggttattgccggaggatatgacttgaagaaccccgagaacattgaacactacgatgaattagtcgagcacatgaaaaagttagaattaccagcggatcagatcgtcttcctgcactctcccagtgatacccaaaaggttaatttaatccgccgttctcgtgctgtactttacaccccggaccgtgaacattttggtatcgtccctgtcgaagcaatgtacttagggacccctgtaattgcggtgaacacggggggaccttgcgagtccgtccgcaacaatgagacgggctttcttgttgatcaaacggcagaggcttttgcggagaaaatgattgacttgatgaaggatgaggaaatgtaccgccgtatgtccgaggaggggccaaaatgggtgcagaaagtgtttgcttttgaggcgtttgcccgtaagctggatgagattatccagtccaccctt

SEQ ID NO: 21 - protein, 400 aa, Caenorhabditis elegans
MVRVTILHPDLGIGGAERLIVDAAVGLQDRGHSVRIFTNQYSRSHCFQETLDLDICTVVPWIPRSIFGKGHALCAYLKMIIAALYIVIYHKDTDVILSDSVSASQFVLRHFSKAKLVFYCHFPDRLLTKRDGNLKAFYRNIIDWIEEYTTGLADVICVNSNFTKNVVRETFKSLASQELTVLYPSLNTEFFDSIEASDDFGEEIPRGTKYVFTSLNRFERKKNIVLALDAFEKLKSNLPADEFSQCHLVIAGGYDLKNPENIEHYDELVEHMKKLELPADQIVFLHSPSDTQKVNLIRRSRAVLYTPDREHFGIVPVEAMYLGTPVIAVNTGGPCESVRNNETGFLVDQTAEAFAEKMIDLMKDEEMYRRMSEEGPKWVQKVFAFEAFARKLDEIIQSTL

SEQ ID NO: 22 - DNA, 1647 bp, Saccharomyces cerevisiae
  source 1..1647: mol_type = other DNA
atgggcagtgcttggacaaactacaattttgaagaggttaagtctcattttgggttcaaaaaatatgttgtatcatctttagtactagtgtatggactaattaaggttctcacgtggatcttccgtcaatgggtgtattccagcttgaatccgttctccaaaaaatcttcattactgaacagagcagttgcctcctgtggtgagaagaatgtgaaagtttttggtttttttcatccgtattgtaatgctggtggtggtggggaaaaagtgctctggaaagctgtagatatcactttgagaaaagatgctaagaacgttattgtcatttattcaggggattttgtgaatggagagaatgttactccggagaatattctaaataatgtgaaagcgaagttcgattacgacttggattcggatagaatatttttcatttcattgaagctaagatacttggtggattcttcaacatggaagcatttcacgttgattggacaagcaattggatcaatgattctcgcatttgaatccattattcagtgtccacctgatatatggattgatacaatggggtaccctttcagctatcctattattgctaggtttttgaggagaattcctatcgtcacatatacgcattatccgataatgtcaaaagacatgttaaataagctgttcaaaatgcccaagaagggtatcaaagtttacggtaaaatattatactggaaagtttttatgttaatttatcaatccattggttctaaaattgatattgtaatcacaaactcaacatggacaaataaccacataaagcaaatttggcaatccaatacgtgtaaaattatatatcctccatgctctactgagaaattagtagattggaagcaaaagtttggtactgcaaagggtgagagattaaatcaagcaattgtgttggcacaatttcgtcctgagaaacgtcataagttaatcattgagtcctttgcaactttcttgaaaaatttaccggattctgtatcgccaattaaattgataatggcggggtccactagatccaagcaagatgaaaattatgttaaaagtttacaagactggtcagaaaatgtattaaaaattcctaaacatttgatatcattcgaaaaaaatctgcccttcgataagattgaaatattactaaacaaatctactttcggtgttaatgccatgtggaatgagcactttggaattgcagttgtagagtatatggcttccggtttgatccccatagttcatgcctcggcgggcccattgttagatatagttactccatgggatgccaacgggaatatcggaaaagctccaccacaatgggagttacaaaagaaatattttgcaaaactcgaagatgatggtgaaactactggatttttctttaaagagccgagtgatcctgattataacacaaccaaagatcctctgagataccctaatttgtccgaccttttcttacaaattacgaaactggactatgactgcctaagggtgatgggcgcaagaaaccagcagtattcattgtataaattctctgatttgaagtttgataaagattgggaaaactttgtactgaatcctatttgtaaattattagaagaggaggaaaggggctga

SEQ ID NO: 23 - protein, 548 aa, Saccharomyces cerevisiae
MGSAWTNYNFEEVKSHFGFKKYVVSSLVLVYGLIKVLTWIFRQWVYSSLNPFSKKSSLLNRAVASCGEKNVKVFGFFHPYCNAGGGGEKVLWKAVDITLRKDAKNVIVIYSGDFVNGENVTPENILNNVKAKFDYDLDSDRIFFISLKLRYLVDSSTWKHFTLIGQAIGSMILAFESIIQCPPDIWIDTMGYPFSYPIIARFLRRIPIVTYTHYPIMSKDMLNKLFKMPKKGIKVYGKILYWKVFMLIYQSIGSKIDIVITNSTWTNNHIKQIWQSNTCKIIYPPCSTEKLVDWKQKFGTAKGERLNQAIVLAQFRPEKRHKLIIESFATFLKNLPDSVSPIKLIMAGSTRSKQDENYVKSLQDWSENVLKIPKHLISFEKNLPFDKIEILLNKSTFGVNAMWNEHFGIAVVEYMASGLIPIVHASAGPLLDIVTPWDANGNIGKAPPQWELQKKYFAKLEDDGETTGFFFKEPSDPDYNTTKDPLRYPNLSDLFLQITKLDYDCLRVMGARNQQYSLYKFSDLKFDKDWENFVLNPICKLLEEEERG

SEQ ID NO: 24 - DNA, 1374 bp, Saccharomyces cerevisiae
  source 1..1374: mol_type = other DNA
atggaaggcgaacagtcacctcagggcgagaagtctctgcagcgcaagcaattcgtgcgtcctcctctggacctgtggcaggacttgaaggacggtgtccgttacgtgatcttcgactgccgtgctaacctgatcgtgatgcccctgctgatcctgttcgagtccatgctgtgcaagatcatcatcaagaaggtggcctacaccgagatcgactacaaggcttacatggaacagatcgagatgatccagctcgacggcatgctggactactcccaagtgtccggtggtactggtcccctggtttaccctgctggtcacgtgctgatctacaagatgatgtactggctgaccgaaggcatggaccacgtcgagaggggtcaagtgttcttccgttacctgtacctgctgaccctggctctgcagatggcttgctactacctgctgcacttgccaccttggtgcgtggtgctggcttgcctgtctaagcgtctgcactccatctacgtgctgcgtctgttcaacgactgcttcaccactctgttcatggtcgtgaccgtgctgggtgctatcgtggcttctcgttgccaccagcgtcctaagctgaagaaatctctggctctggtcatctccgctacctactccatggctgtgtccatcaagatgaacgccctgctgtacttccccgctatgatgatcagcctgttcatcctgaacgacgccaacgtgatcctgactctgctggacctggtcgctatgatcgcttggcaagtggctgtggctgtgcctttcttgcgcagcttccctcagcagtacctgcactgcgctttcaacttcggtcgcaagttcatgtaccagtggtccatcaactggcaaatgatggacgaggaagccttcaacgacaagcgtttccacctcgctctgctgatctcccacctgatcgctctgactaccctgttcgtgactcgttaccctcgtatcctgcctgacctgtggtcctctctgtgtcaccctctccgcaagaacgctgtgctgaacgctaaccccgctaagactatccccttcgtcctgatcgcctccaacttcatcggtgtcctgttctcccgttctctgcactaccagttcttgtcctggtatcactggaccctgcctatcctgatcttttggagcggaatgcccttcttcgtgggtcccatttggtacgtcctgcacgaatggtgctggaactcttaccctcctaactctcaggcttccactctgctgctggctctgaacactgtcctgctgctgctgttggctttgacccagctgtccggttctgtggctctggctaagtcccacctccgtaccacctccagcatggaaaagaagctgaac

SEQ ID NO: 25 - protein, 458 aa, Saccharomyces cerevisiae
MEGEQSPQGEKSLQRKQFVRPPLDLWQDLKDGVRYVIFDCRANLIVMPLLILFESMLCKIIIKKVAYTEIDYKAYMEQIEMIQLDGMLDYSQVSGGTGPLVYPAGHVLIYKMMYWLTEGMDHVERGQVFFRYLYLLTLALQMACYYLLHLPPWCVVLACLSKRLHSIYVLRLFNDCFTTLFMVVTVLGAIVASRCHQRPKLKKSLALVISATYSMAVSIKMNALLYFPAMMISLFILNDANVILTLLDLVAMIAWQVAVAVPFLRSFPQQYLHCAFNFGRKFMYQWSINWQMMDEEAFNDKRFHLALLISHLIALTTLFVTRYPRILPDLWSSLCHPLRKNAVLNANPAKTIPFVLIASNFIGVLFSRSLHYQFLSWYHWTLPILIFWSGMPFFVGPIWYVLHEWCWNSYPPNSQASTLLLALNTVLLLLLALTQLSGSVALAKSHLRTTSSMEKKLN

SEQ ID NO: 26 - DNA, 1833 bp, Homo sapiens
  source 1..1833: mol_type = other DNA
atggcttctagaggcgccagacagagactgaaaggcagcggagctagcagcggagatacagcccctgctgccgataagctgagagagctgctgggatctagagaagccggcggagccgagcacagaacagagctgtctggaaacaaggccggccaagtgtgggcccctgaaggctctacagcctttaagtgcctgctgagcgccagactgtgtgccgctctgctgagcaacatcagcgactgcgacgagacattcaactactgggagcccacacactacctgatctacggcgagggctttcagacctgggagtactctcctgcctacgccatcagaagctacgcctacctgctgctgcatgcctggcctgccgcttttcatgccagaatcctgcagaccaacaagatcctggtgttctacttcctgagatgcctgctggccttcgtgtcctgcatctgcgagctgtacttctacaaggccgtgtgcaagaaattcggcctgcacgtgtcccggatgatgctggcttttctggtgctgagcaccggcatgttctgtagcagcagcgcctttctgcccagctccttctgcatgtacaccacactgatcgccatgaccggctggtacatggacaagacctctatcgccgtgctgggagttgccgctggcgctattcttggctggccattttctgctgccctgggcctgcctatcgccttcgatctgctggtcatgaagcaccggtggaaaagtttcttccactggtccctgatggccctgatcctgttcctggtgcctgtggtggtcatcgacagctactactacggcaagctcgtgatcgcccctctgaacatcgtgctgtacaacgtgttcacccctcacggcccagacctgtatggaaccgagccttggtacttttacctgatcaatggcttcctgaacttcaacgtggccttcgctctggccctgctggttctgcctctgaccagcctgatggaatatctgctgcagcggttccacgtgcagaacctgggacacccttactggctgacactggcccctatgtatatctggttcatcatattcttcattcagccccacaaagaggaacggtttctgttccccgtgtatcccctgatctgcctgtgtggtgctgtggcccttagcgccctgcagaaatgctaccacttcgtgttccagcggtacagactcgagcactacaccgtgacctctaactggctggccctgggcaccgtgtttctgtttggcctgctgtcctttagcagaagcgtggccctgttccggggctatcatggacctctggatctgtaccccgagttctaccggatcgccaccgatcctaccatccacaccgtgcctgaaggcagacccgtgaatgtgtgcgtgggcaaagagtggtacagattcccctccagcttcctgctgcctgacaactggcagctgcaattcatccccagcgagttcagaggccagctgcctaagccttttgccgagggaccactggccaccagaatcgtgcccaccgacatgaacgaccagaatctggaagaacccagccggtacatcgacatcagcaagtgccactacctggtggacctggacaccatgagagagacacccagagagcccaagtacagcagcaacaaagaagagtggatcagcctggcctacagacccttcctggacgcctccagatctagcaagctgctgagggccttctacgtgcccttcctgagcgatcagtacaccgtgtacgtgaactacaccatcctgaagcctcggaaggccaagcagatccggaagaagtctggcgga

SEQ ID NO: 27 - protein, 611 aa, Homo sapiens
MASRGARQRLKGSGASSGDTAPAADKLRELLGSREAGGAEHRTELSGNKAGQVWAPEGSTAFKCLLSARLCAALLSNISDCDETFNYWEPTHYLIYGEGFQTWEYSPAYAIRSYAYLLLHAWPAAFHARILQTNKILVFYFLRCLLAFVSCICELYFYKAVCKKFGLHVSRMMLAFLVLSTGMFCSSSAFLPSSFCMYTTLIAMTGWYMDKTSIAVLGVAAGAILGWPFSAALGLPIAFDLLVMKHRWKSFFHWSLMALILFLVPVVVIDSYYYGKLVIAPLNIVLYNVFTPHGPDLYGTEPWYFYLINGFLNFNVAFALALLVLPLTSLMEYLLQRFHVQNLGHPYWLTLAPMYIWFIIFFIQPHKEERFLFPVYPLICLCGAVALSALQKCYHFVFQRYRLEHYTVTSNWLALGTVFLFGLLSFSRSVALFRGYHGPLDLYPEFYRIATDPTIHTVPEGRPVNVCVGKEWYRFPSSFLLPDNWQLQFIPSEFRGQLPKPFAEGPLATRIVPTDMNDQNLEEPSRYIDISKCHYLVDLDTMRETPREPKYSSNKEEWISLAYRPFLDASRSSKLLRAFYVPFLSDQYTVYVNYTILKPRKAKQIRKKSGG

SEQ ID NO: 28 - DNA, 1470 bp, Gallus gallus
  source 1..1470: mol_type = other DNA
atggcccagaagagaagcagcagcggcagaagctttcccctgctgctgctgatcatcgtggtggcctttgtgcacctgaccgtgtgtcccttcaccaaggtggaagagagcttcaacctgcaagccatccacgacgtggtgtaccaccagctggacctggataagtacgaccaccacgagttccctggcgtggtgcccagaacttttctgggccccatctttatcgccgctctgagcagccctgccatctacatcctgagcctgctgaagatgagcaagttctacagccagctgatcgtgcggggctctctgggactgagcgtgatctacacactgtggaagctgcagaaagaagtgcggaagcagttcggcgccaccaccagcacagtgttctgcctgatcaccgtgacacagttccacctgatgttctactgcacccggacactgcccaacgtgttcgccctgccttttgtgctgctggccctgaccttctggattcagcagaagcagcggcccttcatctggttttctgccctggccatcatcgtgttcagaagcgagctggccatcttcctgggcctgatgctgctggtcaccttcctgaccaagcggatcagcgtgctgaaaatcctgtctcacgccgtgcctgccggcttcttttggctgggacttacagtggccgtggacagcctgttttggagacagctcgtttggcccgagggcaaagtgctgtggtacaacaccatcctgaacaagagcagcaactggggcacaagcccctttttctggtacttctacagcgccctgccacgcgctctgggctgttctattgtgttcgtgcctctgggagccgccgagaagagaaccagaattctcctgctgcctgctctgggttttatcttcctgtacagcttcctgcctcacaaagagctgcggttcatcatctacacattccccgtgttcaacatcgtggccgccaaagtgtgcagccggattctgaacaactaccggaagtcctggctgtacaagctgggcagcctgttcgtggtcatgcatctgctggttaacgccgcctacagcggcaccagcctgtacgtgtcccacttcaattatcctggcggcgtggccatccagaaactgcacgaactggtgcctagcaccgccgaagtgtccgtgcacattgatgtggctgctgcccagacaggcgtgtccagattcctggaaatcaacagcgattggcgctacgacaagcgcgaggatgtgaagcctggcgaccagctgatgttcagctacacccacatcctgatggaaacaaaccctctgcagatcagccactacaagaccacacacagacccctggccaacattcccggcatctctaagatcggcctgaacctgacagctctgcctcctttcacactgaatctgaagcccaagctggtgctgctcgagaagctgcctctcagctct

SEQ ID NO: 29 - protein, 490 aa, Gallus gallus
MAQKRSSSGRSFPLLLLIIVVAFVHLTVCPFTKVEESFNLQAIHDVVYHQLDLDKYDHHEFPGVVPRTFLGPIFIAALSSPAIYILSLLKMSKFYSQLIVRGSLGLSVIYTLWKLQKEVRKQFGATTSTVFCLITVTQFHLMFYCTRTLPNVFALPFVLLALTFWIQQKQRPFIWFSALAIIVFRSELAIFLGLMLLVTFLTKRISVLKILSHAVPAGFFWLGLTVAVDSLFWRQLVWPEGKVLWYNTILNKSSNWGTSPFFWYFYSALPRALGCSIVFVPLGAAEKRTRILLLPALGFIFLYSFLPHKELRFIIYTFPVFNIVAAKVCSRILNNYRKSWLYKLGSLFVVMHLLVNAAYSGTSLYVSHFNYPGGVAIQKLHELVPSTAEVSVHIDVAAAQTGVSRFLEINSDWRYDKREDVKPGDQLMFSYTHILMETNPLQISHYKTTHRPLANIPGISKIGLNLTALPPFTLNLKPKLVLLEKLPLSS

SEQ ID NO: 30 - DNA, 1059 bp, Pyrococcus furiosus
  source 1..1059: mol_type = other DNA
atgaaagtgagcgttattatcccgacctataatgaacgtgaaaacctggaagaactgtttagccgtattgataatgcactgcagggtctgaattatgaaattgttgttgtggatgatgatagtccggatcgtacctgggaaaaagcacaagaactgagcagcaaatatccggttaaagttattcgtcgcaccaaagaaaaaggtctgagcagcgcagtgattcgtggttttaaagaagcatcaggcgacgtttttgttgtgatggatgccgatctgcagcatccgcctgaagttattccgaaactgattgaagccattaaaaacggtagcgatattgcaattggtagccgttatgttaaaggtggcaaagttgaaaactggccgttttatcgtaaactgattagcaaaggtgccattatggttggtcgtattgcactgccgaaaattcgcgatattaaagatccggttagcggtttttttgccctgcgtaaagaagttgttgaaggcgttgaactgaatccgattggctttaaaatcctgatggaaattctgatcaaaggcaagtatagcaaagttgtggaagtgccgtttacctttggtattcgtgcacgtggtgaaagcaaactgaaaggcaaaaccatctttgaatatctgcgccatatttaccgtctgatgaaatgggaaggtgaaattgatcgcatcgtgaaatttagcattgttggtctgagcggtattctggtgaatgaaggttttctgtggctgtttgttaatctgggcattccgaaagaaattgccgttattccggcagttgaactgtcaattctgaacaactttttctggaacgatatctggaccttcaaagatattcgccgtggtagcatttttagtcgcctgctgaaattccatattgcagcactgagcggtgcagttgttaactttattgtttattggatcctgctgtttctgggcatccattatctgattgcaaatctggttggtatcgttctgagctttggtgttcgttatgtgattaatcgtcatgttacctgggcaacctaa

SEQ ID NO: 31 - protein, 352 aa, Pyrococcus furiosus
MKVSVIIPTYNERENLEELFSRIDNALQGLNYEIVVVDDDSPDRTWEKAQELSSKYPVKVIRRTKEKGLSSAVIRGFKEASGDVFVVMDADLQHPPEVIPKLIEAIKNGSDIAIGSRYVKGGKVENWPFYRKLISKGAIMVGRIALPKIRDIKDPVSGFFALRKEVVEGVELNPIGFKILMEILIKGKYSKVVEVPFTFGIRARGESKLKGKTIFEYLRHIYRLMKWEGEIDRIVKFSIVGLSGILVNEGFLWLFVNLGIPKEIAVIPAVELSILNNFFWNDIWTFKDIRRGSIFSRLLKFHIAALSGAVVNFIVYWILLFLGIHYLIANLVGIVLSFGVRYVINRHVTWAT

SEQ ID NO: 32 - protein, 6 aa, synthetic construct
  SITE 1: note = fluorescently-labelled with 5-Carboxytetramethylrhodamine (TAMRA)
YANATS

SEQ ID NO: 33 - protein, 10 aa, synthetic construct
  SITE 1: note = fluorescently labelled with 5-carboxyfluorescein
GSDANYTYTQ

SEQ ID NO: 34 - protein, 8 aa, synthetic construct
  SITE 1: note = fluorescently labelled with 5-carboxyfluorescein
GSLANYTK

SEQ ID NO: 35 - DNA, 1254 bp, Saccharomyces cerevisiae
  source 1..1254: mol_type = other DNA
ggcaacaagtcgaccaaaaaaaggatcatcatatttgtgctgggtgatgtaggacactctccaaggatatgctatcacgctataagtttcagtaagttaggttggcaagtcgagctatgcggttatgtggaggacactctacccaaaattatttccagtgatccaaatatcaccgtccatcatatgtcaaacttgaaaagaaagggaggcggaacatcagttatatttatggtaaagaaggtgctttttcaagttttaagtattttcaaattactttgggaattgagaggaagcgattacatactagttcaaaatccaccgagcatacccattcttccgattgctgtgctatacaagttgaccggttgtaaactaattattgattggcacaatctagcatattcgatattgcaactaaaatttaaaggaaacttttaccatcctttagtgttgatatcttacatggtagagatgatattcagcaaatttgctgattataacttgactgttactgaagcaatgaggaaatatttaattcaaagctttcacttgaatccaaagagatgtgctgttctctacgaccgcccggcttcccaatttcaacctttggcaggtgacatttctcgtcaaaaagccctaactaccaaagcctttataaagaattatattcgcgatgattttgatacagaaaaaggcgataaaattattgtgacttcaacatcattcacccctgatgaagatattggtattttattaggtgccctaaagatttacgaaaactcttatgtcaaatttgattcaagtttgcctaagatcttgtgttttataacgggtaaaggaccactaaaggagaaatatatgaagcaagtagaagaatatgactggaagcgctgtcaaatcgaatttgtgtggttgtcagcagaggattacccaaagttattacaattatgcgattacggagtttccctgcatacttcaagttcagggttggacctgccaatgaaaattttagatatgtttggctcaggtcttcctgttattgcaatgaactatccagtgcttgacgaattagtacaacacaatgtaaatgggttaaaatttgttgatagaagggagcttcatgaatctctgatttttgctatgaaagatgctgatttataccaaaaattgaagaaaaatgtaacgcaggaagctgagaacagatggcaatcaaattgggaacgaacaatgagagatttgaagctaattcattga

SEQ ID NO: 36 - protein, 417 aa, Saccharomyces cerevisiae
GNKSTKKRIIIFVLGDVGHSPRICYHAISFSKLGWQVELCGYVEDTLPKIISSDPNITVHHMSNLKRKGGGTSVIFMVKKVLFQVLSIFKLLWELRGSDYILVQNPPSIPILPIAVLYKLTGCKLIIDWHNLAYSILQLKFKGNFYHPLVLISYMVEMIFSKFADYNLTVTEAMRKYLIQSFHLNPKRCAVLYDRPASQFQPLAGDISRQKALTTKAFIKNYIRDDFDTEKGDKIIVTSTSFTPDEDIGILLGALKIYENSYVKFDSSLPKILCFITGKGPLKEKYMKQVEEYDWKRCQIEFVWLSAEDYPKLLQLCDYGVSLHTSSSGLDLPMKILDMFGSGLPVIAMNYPVLDELVQHNVNGLKFVDRRELHESLIFAMKDADLYQKLKKNVTQEAENRWQSNWERTMRDLKLIH

SEQ ID NO: 37 - DNA, 1512 bp, Saccharomyces cerevisiae
  source 1..1512: mol_type = other DNA
tattccagcttgaatccgttctccaaaaaatcttcattactgaacagagcagttgcctcctgtggtgagaagaatgtgaaagtttttggtttttttcatccgtattgtaatgctggtggtggtggggaaaaagtgctctggaaagctgtagatatcactttgagaaaagatgctaagaacgttattgtcatttattcaggggattttgtgaatggagagaatgttactccggagaatattctaaataatgtgaaagcgaagttcgattacgacttggattcggatagaatatttttcatttcattgaagctaagatacttggtggattcttcaacatggaagcatttcacgttgattggacaagcaattggatcaatgattctcgcatttgaatccattattcagtgtccacctgatatatggattgatacaatggggtaccctttcagctatcctattattgctaggtttttgaggagaattcctatcgtcacatatacgcattatccgataatgtcaaaagacatgttaaataagctgttcaaaatgcccaagaagggtatcaaagtttacggtaaaatattatactggaaagtttttatgttaatttatcaatccattggttctaaaattgatattgtaatcacaaactcaacatggacaaataaccacataaagcaaatttggcaatccaatacgtgtaaaattatatatcctccatgctctactgagaaattagtagattggaagcaaaagtttggtactgcaaagggtgagagattaaatcaagcaattgtgttggcacaatttcgtcctgagaaacgtcataagttaatcattgagtcctttgcaactttcttgaaaaatttaccggattctgtatcgccaattaaattgataatggcggggtccactagatccaagcaagatgaaaattatgttaaaagtttacaagactggtcagaaaatgtattaaaaattcctaaacatttgatatcattcgaaaaaaatctgcccttcgataagattgaaatattactaaacaaatctactttcggtgttaatgccatgtggaatgagcactttggaattgcagttgtagagtatatggcttccggtttgatccccatagttcatgcctcggcgggcccattgttagatatagttactccatgggatgccaacgggaatatcggaaaagctccaccacaatgggagttacaaaagaaatattttgcaaaactcgaagatgatggtgaaactactggatttttctttaaagagccgagtgatcctgattataacacaaccaaagatcctctgagataccctaatttgtccgaccttttcttacaaattacgaaactggactatgactgcctaagggtgatgggcgcaagaaaccagcagtattcattgtataaattctctgatttgaagtttgataaagattgggaaaactttgtactgaatcctatttgtaaattattagaagaggaggaaaggggctga

SEQ ID NO: 38 - protein, 503 aa, Saccharomyces cerevisiae
YSSLNPFSKKSSLLNRAVASCGEKNVKVFGFFHPYCNAGGGGEKVLWKAVDITLRKDAKNVIVIYSGDFVNGENVTPENILNNVKAKFDYDLDSDRIFFISLKLRYLVDSSTWKHFTLIGQAIGSMILAFESIIQCPPDIWIDTMGYPFSYPIIARFLRRIPIVTYTHYPIMSKDMLNKLFKMPKKGIKVYGKILYWKVFMLIYQSIGSKIDIVITNSTWTNNHIKQIWQSNTCKIIYPPCSTEKLVDWKQKFGTAKGERLNQAIVLAQFRPEKRHKLIIESFATFLKNLPDSVSPIKLIMAGSTRSKQDENYVKSLQDWSENVLKIPKHLISFEKNLPFDKIEILLNKSTFGVNAMWNEHFGIAVVEYMASGLIPIVHASAGPLLDIVTPWDANGNIGKAPPQWELQKKYFAKLEDDGETTGFFFKEPSDPDYNTTKDPLRYPNLSDLFLQITKLDYDCLRVMGARNQQYSLYKFSDLKFDKDWENFVLNPICKLLEEEERG